European Patent Application EP 4 775 589 A1, published July 15, 2026. Title: COMPOSICIÓN FARMACÉUTICA QUE COMPRENDE UN PÉPTIDO O UNA COMBINACIÓN DE PÉPTIDOS AGONISTAS DE LOS RECEPTORES MAS, AT1 Y AT2. Applicant: PONTIFICIA UNIVERSIDAD CATÓLICA DE CHILE. Application IB PCT/CL2023/050084, filed September 8, 2023. The sequence listing filed with the application follows.

SEQUENCE LISTING (3 sequences)

SEQ ID NO: 1 - protein, 16 aa, synthetic construct
  SITE 1: note = D-histidine
  SITE 2: note = D-phenylalanine
  SITE 3: note = D-proline
  SITE 4: note = D-histidine
  SITE 5: note = D-isoleucine
  SITE 6: note = D-tyrosine
  SITE 7: note = D-valine
  SITE 8: note = D-arginine
  SITE 9: note = D-aspartic acid
HFPHIYVRDDRVYIHP

SEQ ID NO: 2 - protein, 9 aa, synthetic construct
  SITE 1: note = D-histidine
  SITE 2: note = D-phenylalanine
  SITE 3: note = D-proline
  SITE 4: note = D-histidine
  SITE 5: note = D-isoleucine
  SITE 6: note = D-tyrosine
  SITE 7: note = D-valine
  SITE 8: note = D-arginine
  SITE 9: note = D-aspartic acid
HFPHIYVRD

SEQ ID NO: 3 - protein, 7 aa, synthetic construct
DRVYIHP